European Patent Application EP 4 796 639 A1, published August 26, 2026. Title: RNA structures for improving protein translation efficiency, mRNA structures comprising the same, and uses thereof. Applicant: Korea Research Institute of Bioscience and Biotechnology. Application KR. The sequence listing filed with the application follows.

SEQUENCE LISTING (17 sequences)

SEQ ID NO: 1 - RNA, 81 nt, synthetic construct
  source 1..81: mol_type = other RNA
tttgcaggcagcggaaccccccacctggcgacaggtgcctctgcggccaaaagccacgtgtataagatacacctgcaaagg

SEQ ID NO: 2 - RNA, 121 nt, synthetic construct
  source 1..121: mol_type = other RNA
cttcgatgcgttgcgctcagcactcaaccccagagtgtagcttaggctgatgagtctggacatccctcaccggtgacggtggtccaggctgcgttggcggcctacctatggctaacgccat

SEQ ID NO: 3 - RNA, 101 nt, synthetic construct
  source 1..101: mol_type = other RNA
gcggctaatcccaacctcggagcaggtggtcacaaaccagtgattggcctgtcgtaacgcgcaagtccgtggcggaaccgactactttgggtgtccgtgtt

SEQ ID NO: 4 - RNA, 76 nt, synthetic construct
  source 1..76: mol_type = other RNA
tggtggccgtgggaactcctccttggtaacaaggacccacggggccgaaagccacgtcctgacggacccaccatgt

SEQ ID NO: 5 - RNA, 114 nt, synthetic construct
  source 1..114: mol_type = other RNA
tgcttcgtagcggagcatggtggccgtgggaactcctccttggtaacaaggacccacggggccgaaagccacgtcctgacggacccaccatgtgtgcaaccccagcacggcaac

SEQ ID NO: 6 - RNA, 102 nt, synthetic construct
  source 1..102: mol_type = other RNA
ttcaggtaccccgaggtaacacgcgacactcgggatctgagaaggggactggggcttctgtaaaagcgcccagtttaaaaagcttctatgcctggataggtg

SEQ ID NO: 7 - RNA, 94 nt, synthetic construct
  source 1..94: mol_type = other RNA
gcggaaccggtgagtacaccggaattgccaggacgaccgggtcctttcttggataaacccgctcaatgcctggagatttgggcgtgcccccgca

SEQ ID NO: 8 - RNA, 53 nt, synthetic construct
  source 1..53: mol_type = other RNA
acatttgcttctgacatagttgtgttgactcacaaccccagaaacagacatcc

SEQ ID NO: 9 - RNA, 215 nt, synthetic construct
  source 1..215: mol_type = other RNA
gcctcgactgtgccttctagttgccagccatctgttgtttgcccctcccccgtgccttccttgaccctggaaggtgccactcccactgtcctttcctaataaaatgaggaaattgcatcgcattgtctgagtaggtgtcattctattctggggggtggggtggggcaggacagcaagggggaggattgggaagacaatagcaggcatgctgggga

SEQ ID NO: 10 - RNA, 786 nt, synthetic construct
  source 1..786: mol_type = other RNA
atggtgagcaagggcgccgagctgttcaccggcatcgtgcccatcctgatcgagctgaatggcgatgtgaatggccacaagttcagcgtgagcggcgagggcgagggcgatgccacctacggcaagctgaccctgaagttcatctgcaccaccggcaagctgcctgtgccctggcccaccctggtgaccaccctgagctacggcgtgcagtgcttctcacgctaccccgatcacatgaagcagcacgacttcttcaagagcgccatgcctgagggctacatccaggagcgcaccatcttcttcgaggatgacggcaactacaagtcgcgcgccgaggtgaagttcgagggcgataccctggtgaatcgcatcgagctgaccggcaccgatttcaaggaggatggcaacatcctgggcaataagatggagtacaactacaacgcccacaatgtgtacatcatgaccgacaaggccaagaatggcatcaaggtgaacttcaagatccgccacaacatcgaggatggcagcgtgcagctggccgaccactaccagcagaatacccccatcggcgatggccctgtgctgctgcccgataaccactacctgtccacccagagcgccctgtccaaggaccccaacgagaagcgcgatcacatgatctacttcggcttcgtgaccgccgccgccatcacccacggcatggatgagctgtacaagtccggactcagatctcgagctcaagcttcgaattctgcagtcgacggtaccgcgggcccgggatcctaa

SEQ ID NO: 11 - RNA, 1191 nt, synthetic construct
  source 1..1191: mol_type = other RNA
atggcattaccagtgaccgccttgctcctgccgctggccttactgctccacgccgccaggccggcggcccagccggccgtggacaacaagtttaataaggagatgtgggccgcttgggaggaaatccgaaatctcccgaatctgaacgggtggcagatgacggcttttatcgcatcacttgtggacgacccatcccaatctgctaatctcttggcggaggcgaagaaattgaacgacgctcaagcgcccaaaggcccgggaggccgcgaacaaaaactcatctcagaagaggatctgaagcttggggtcaccgtctcttcagcgctgagcaactccatcatgtacttcagccacttcgtgccggtcttcctgccagcgaagcccaccacgacgccagcgccgcgaccaccaacaccggcgcccaccatcgcgtcgcagcccctgtccctgcgcccagaggcatgccggccagcggcggggggcgcagtgcacacgagggggctggataagcttgtgaaagggaaacacctttgtccaagtcccctatttcccggaccttctaagcccttttgggtgctggtggtggttggtggagtcctggcttgctatagcttgctagtaacagtggcctttattattttctgggtgaggagtaagaggagcaggctcctgcacagtgactacatgaacatgactccccgccgccccgggcccacccgcaagcattaccagccctatgccccaccacgcgacttcgcagcctatgaattcctgtgcgcacgcccacgccgcagccccgcccaagaagatggcaaagtctacatcaacatgccaggcaggggcgcggccgctagagtgaagttcagcaggagcgcagacgcccccgcgtaccagcagggccagaaccagctctataacgagctcaatctaggacgaagagaggagtacgatgttttggacaagagacgtggccgggaccctgagatggggggaaagccgagaaggaagaaccctcaggaaggcctgtacaatgaactgcagaaagataagatggcggaggcctacagtgagattgggatgaaaggcgagcgccggaggggcaaggggcacgatggcctttaccagggtctcagtacagccaccaaggacacctacgacgcccttcacatgcaggccctgccccctcgctaa

SEQ ID NO: 12 - RNA, 3825 nt, synthetic construct
  source 1..3825: mol_type = other RNA
atgttcgtgttcctggtgctgctgcctctggtgtccagccagtgtgtgaacctgaccaccagaacacagctgcctccagcctacaccaacagctttaccagaggcgtgtactaccccgacaaggtgttcagatccagcgtgctgcactctacccaggacctgttcctgcctttcttcagcaacgtgacctggttccacgccatccacgtgtccggcaccaatggcaccaagagattcgacaaccccgtgctgcccttcaacgacggggtgtactttgccagcaccgagaagtccaacatcatcagaggctggatcttcggcaccacactggacagcaagacccagagcctgctgatcgtgaacaacgccaccaacgtggtcatcaaagtgtgcgagttccagttctgcaacgaccccttcctgggcgtctactaccacaagaacaacaagagctggatggaaagcgagttccgggtgtacagcagcgccaacaactgcaccttcgagtacgtgtcccagcctttcctgatggacctggaaggcaagcagggcaacttcaagaacctgcgcgagttcgtgtttaagaacatcgacggctacttcaagatctacagcaagcacacccctatcaacctcgtgcgggatctgcctcagggcttctctgctctggaacccctggtggatctgcccatcggcatcaacatcacccggtttcagacactgctggccctgcacagaagctacctgacacctggcgatagcagcagcggatggacagctggtgccgccgcttactatgtgggctacctgcagcctagaaccttcctgctgaagtacaacgagaacggcaccatcaccgacgccgtggattgtgctctggatcctctgagcgagacaaagtgcaccctgaagtccttcaccgtggaaaagggcatctaccagaccagcaacttccgggtgcagcccaccgaatccatcgtgcggttccccaatatcaccaatctgtgccccttcggcgaggtgttcaatgccaccagattcgcctctgtgtacgcctggaaccggaagcggatcagcaattgcgtggccgactactccgtgctgtacaactccgccagcttcagcaccttcaagtgctacggcgtgtcccctaccaagctgaacgacctgtgcttcacaaacgtgtacgccgacagcttcgtgatccggggagatgaagtgcggcagattgcccctggacagacaggcaagatcgccgactacaactacaagctgcccgacgacttcaccggctgtgtgattgcctggaacagcaacaacctggactccaaagtcggcggcaactacaattacctgtaccggctgttccggaagtccaatctgaagcccttcgagcgggacatctccaccgagatctatcaggccggcagcaccccttgtaacggcgtggaaggcttcaactgctacttcccactgcagtcctacggctttcagcccacaaatggcgtgggctatcagccctacagagtggtggtgctgagcttcgaactgctgcatgcccctgccacagtgtgcggccctaagaaaagcaccaatctcgtgaagaacaaatgcgtgaacttcaacttcaacggcctgaccggcaccggcgtgctgacagagagcaacaagaagttcctgccattccagcagtttggccgggatatcgccgataccacagacgccgttagagatccccagacactggaaatcctggacatcaccccttgcagcttcggcggagtgtctgtgatcacccctggcaccaacaccagcaatcaggtggcagtgctgtaccaggacgtgaactgtaccgaagtgcccgtggccattcacgccgatcagctgacacctacatggcgggtgtactccaccggcagcaatgtgtttcagaccagagccggctgtctgatcggagccgagcacgtgaacaatagctacgagtgcgacatccccatcggcgctggaatctgcgccagctaccagacacagacaaacagccctcggagagccagaagcgtggccagccagagcatcattgcctacacaatgtctctgggcgccgagaacagcgtggcctactccaacaactctatcgctatccccaccaacttcaccatcagcgtgaccacagagatcctgcctgtgtccatgaccaagaccagcgtggactgcaccatgtacatctgcggcgattccaccgagtgctccaacctgctgctgcagtacggcagcttctgcacccagctgaatagagccctgacagggatcgccgtggaacaggacaagaacacccaagaggtgttcgcccaagtgaagcagatctacaagacccctcctatcaaggacttcggcggcttcaatttcagccagattctgcccgatcctagcaagcccagcaagcggagcttcatcgaggacctgctgttcaacaaagtgacactggccgacgccggcttcatcaagcagtatggcgattgtctgggcgacattgccgccagggatctgatttgcgcccagaagtttaacggactgacagtgctgcctcctctgctgaccgatgagatgatcgcccagtacacatctgccctgctggccggcacaatcacaagcggctggacatttggagcaggcgccgctctgcagatcccctttgctatgcagatggcctaccggttcaacggcatcggagtgacccagaatgtgctgtacgagaaccagaagctgatcgccaaccagttcaacagcgccatcggcaagatccaggacagcctgagcagcacagcaagcgccctgggaaagctgcaggacgtggtcaaccagaatgcccaggcactgaacaccctggtcaagcagctgtcctccaacttcggcgccatcagctctgtgctgaacgatatcctgagcagactggaccctcctgaggccgaggtgcagatcgacagactgatcacaggcagactgcagagcctccagacatacgtgacccagcagctgatcagagccgccgagattagagcctctgccaatctggccgccaccaagatgtctgagtgtgtgctgggccagagcaagagagtggacttttgcggcaagggctaccacctgatgagcttccctcagtctgcccctcacggcgtggtgtttctgcacgtgacatatgtgcccgctcaagagaagaatttcaccaccgctccagccatctgccacgacggcaaagcccactttcctagagaaggcgtgttcgtgtccaacggcacccattggttcgtgacacagcggaacttctacgagccccagatcatcaccaccgacaacaccttcgtgtctggcaactgcgacgtcgtgatcggcattgtgaacaataccgtgtacgaccctctgcagcccgagctggacagcttcaaagaggaactggacaagtactttaagaaccacacaagccccgacgtggacctgggcgatatcagcggaatcaatgccagcgtcgtgaacatccagaaagagatcgaccggctgaacgaggtggccaagaatctgaacgagagcctgatcgacctgcaagaactggggaagtacgagcagtacatcaagtggccctggtacatctggctgggctttatcgccggactgattgccatcgtgatggtcacaatcatgctgtgttgcatgaccagctgctgtagctgcctgaagggctgttgtagctgtggcagctgctgcaagttcgacgaggacgattctgagcccgtgctgaagggcgtgaaactgcactacacatgatga

SEQ ID NO: 13 - RNA, 580 nt, synthetic construct
  source 1..580: mol_type = other RNA
tccccctctccctccccccccccctaacgttactggccgaagccgcttggaataaggccggtgtgcgtttgtctatatgttattttccaccatattgccgtcttttggcaatgtgagggcccggaaacctggccctgtcttcttgacgagcattcctaggggtctttcccctctcgccaaaggaatgcaaggtctgttgaatgtcgtgaaggaagcagttcctctggaagcttcttgaagacaaacaacgtctgtagcgaccctttgcaggcagcggaaccccccacctggcgacaggtgcctctgcggccaaaagccacgtgtataagatacacctgcaaaggcggcacaaccccagtgccacgttgtgagttggatagttgtggaaagagtcaaatggctctcctcaagcgtattcaacaaggggctgaaggatgcccagaaggtaccccattgtatgggatctgatctggggcctcggtgcacatgctttacatgtgtttagtcgaggttaaaaaacgtctaggccccccgaaccacggggacgtggttttcctttgaaaaacacgttgataatttg

SEQ ID NO: 14 - RNA, 91 nt, synthetic construct
  source 1..91: mol_type = other RNA
gcctcgactgtgccttctagttgccagccatctgttgtttgcccctcccccgtgccttccttgaccctggaaggtgccactcccactgtcc

SEQ ID NO: 15 - RNA, 55 nt, synthetic construct
  source 1..55: mol_type = other RNA
gcctcgactgtgccttctagttgccagccatctgttgtttgcccctcccccgtgc

SEQ ID NO: 16 - RNA, 36 nt, synthetic construct
  source 1..36: mol_type = other RNA
gcctcgactgtgccttctagttgccagccatctgtt

SEQ ID NO: 17 - RNA, 18 nt, synthetic construct
  source 1..18: mol_type = other RNA
gcctcgactgtgccttct